European Patent Specification EP 3 296 403 B1, published April 1, 2026. Title: Soybean Transgenic Event MON87751 and Methods for Detection and Use Thereof. Applicant: Monsanto Technology LLC. The sequence listing filed with the application follows.

SEQUENCE LISTING (26 sequences)

SEQ ID NO: 1 - DNA, 20 bp, Artificial Sequence
  Artificial DNA sequence comprising soybean genomic sequence and transgene sequence
ttggagatctccagtcagca

SEQ ID NO: 2 - DNA, 20 bp, Artificial Sequence
  Artificial DNA sequence comprising soybean genomic sequence and transgene sequence
catgtagattcctatgagaa

SEQ ID NO: 3 - DNA, 60 bp, Artificial Sequence
  Artificial DNA sequence comprising soybean genomic sequence and transgene sequence
tgtagatatttcccctcactttggagatctccagtcagcatcatcacaccaaaagttagg

SEQ ID NO: 4 - DNA, 60 bp, Artificial Sequence
  Artificial DNA sequence comprising soybean genomic sequence and transgene sequence
catcatactcattgctgatccatgtagattcctatgagaatgagaggacaagacagctcg

SEQ ID NO: 5 - DNA, 100 bp, Artificial Sequence
  Artificial DNA sequence comprising soybean genomic sequence and transgene sequence
ttgctctttggagtttattttgtagatatttcccctcactttggagatctccagtcagcatcatcacaccaaaagttaggcccgaatagtttgaaattag

SEQ ID NO: 6 - DNA, 100 bp, Artificial Sequence
  Artificial DNA sequence comprising soybean genomic sequence and transgene sequence
ttctttttctccatattgaccatcatactcattgctgatccatgtagattcctatgagaatgagaggacaagacagctcggtcaaaactcaatcgtcgaa

SEQ ID NO: 7 - DNA, 1626 bp, Artificial Sequence
  Artificial DNA sequence comprising soybean genomic sequence and transgene sequence
ttaatttttaagtaaactaatttatgtctaaagggtttattttaaaaataggttaataataaaatttcatatgatttttttatcaaacacaaaaattatttaaaattaatttaaatttaaattaattttagactaaaaaataatttatcaatatgaagcctaatatgtgaatattaccctatatttacatcttaagtatgtgagttaggtttactaatattatatttcataggtcttttttgttgattttatacatatttcttttcatataaataataacgtttttttatcgtaattattaattttttatttttattaacaggaattcgaagtcatatttatttctttctcgtttagatagcaacttaatgttatgtatttccgttaatacatttttaaaaaaatttacgatattatgataagtcatgatcaaatacgaaacatacttagtgtaacgtcattaaattccatttccatggaatgtgagtacagttcattatttaatttaattttttttttgttgcagaatttaattgaccaggttttgtggtgacgtctctgcacaggcttcccgtaaggcgtcctaatcataatcttaaaattcttcaatatctaccttgtattttgggtaatgggaaaatcagactcgatctgtattttcagttgcaattctcttccttctcgtgactctccagtaccttgttgatttgaacgacttggttaatctttaaattaccttcattaaacattcgtttgaattaggtgttacattgttaggaccacaacggtgtgacctcacaaccttgcggagttaattatggtggattggtgggtacatatatagactcatcatcaggaacaaaaaatatctacgaaaccattatatttatttttgttgtttgagactgtctacatgaatgatacgagactaaagattgttatttgtcaggaattgtaatttatttttactacaatataaacaacgagaaaaacaacggttaggttgacatggtaatcaactaattgtatttaaaaaaaaaaaaaaaaacaattgtaccatcgtacttggctcatgagatccccacatgcttagatcagggcaatccttaactatcactcatgaactcagtcacgacacatagaggaatagttagcgaatgtgactcgaacattgcacgactcccatgacacctgatatgtatatatagatccagatgagagactcacacgtacattttactcatcccaattataaatacataaacactatagaacaccactaaattgctctttggagtttattttgtagatatttcccctcactttggagatctccagtcagcatcatcacaccaaaagttaggcccgaatagtttgaaattagaaagctcgcaattgaggtctgtcgaccctgcaggtacactggcgcgccacctcagcgctgtgcctgttgcgacaactatttttatgtatgcaagagtcagcatatgtataattgattcagaatcgttttgacgagttcggatgtagtagtagccattatttaatgtacatactaatcgtgaatagtgaatatgatgaaacattgtatcttattgtataaatatccataaacacatcatgaaa

SEQ ID NO: 8 - DNA, 1452 bp, Artificial Sequence
  Artificial DNA sequence comprising soybean genomic sequence and transgene sequence
cgcatcgatcgtgaagtttctcatctaagcccccatttggacgtgaatgtagacacgtcgaaataaagatttccgaattagaataatttgtttattgctttcgcctataaatacgacggatcgtaatttgtcgttttatcaaaatgtactttcattttataataacgctgcggacatctacatttttgaattgaaaaaaaattggtaattactctttctttttctccatattgaccatcatactcattgctgatccatgtagattcctatgagaatgagaggacaagacagctcggtcaaaactcaatcgtcgaaattcaatgggaacattttggtatctaacctcaacttcaatactggagatcggaaattccactaacaaggaaatgaccattcgatcggacctcatcagaactcagtagtaacatattgtatttgaaagaacaattaaatcatatataagcttttgtggaaaaaaaggatactacgtactaaaatataaacgttgaagtaaattacagaaaatgctaatttcataacacggttatcttcaaattttagtggcccgtttaagccctagttaaatcaaatatatgaatgcagtttatgtataaggtatgcatgtgttatagttaatcgagtttagataattagaatcaaatatatgattaatggtacctgtgttacataaagagactaattaacctaagttctgaacaagtaattaatcaaacattgaagtgatagatgttgggcctaaatccagagcataacctttacgtcaatgaactacaaattttcacactagaaacatacattgaactttttttccttcgtttaaactccttttcttttaactgtgtttccgcgtttaatcaaattttacgtgtgtcgaccgaaagttagaaattataactaataacagactcaagttgacgtaattttttcatgatacctacgtattgctcggagtttagatgctatataaacatgagtgatgacatggttttaaattgtgcttccagttgtgttaccatgaactaaaaaatcttataggtaattgtaagaaaatatgattgatccagtcatgattgcggttatgatgcgattgtacagaatcaaaataccttgaaattgcgattgcaattgttattacagactccaatttaaaatcatgagtgaggattttatgatagatcgaatcaatgtttcacactacacctggaataaaaacctgagtcgtttattagatctatatcttcatatgcatgcatgtaccttagctattcatttttcactgtaaatctttactcacacttaaaatagtcgtgcatttgatatttgaatgaaatttatagagctttcgatttgagatagtcccatctctatttgggttggtcaatcatggagcatgaaaaaaacaatagtttagctaggccaggccaaattaat

SEQ ID NO: 9 - DNA, 10119 bp, Artificial Sequence
  Artificial DNA sequence comprising transgene sequence
ccagtcagcatcatcacaccaaaagttaggcccgaatagtttgaaattagaaagctcgcaattgaggtctgtcgaccctgcaggtacactggcgcgccacctcagcgctgtgcctgttgcgacaactatttttatgtatgcaagagtcagcatatgtataattgattcagaatcgttttgacgagttcggatgtagtagtagccattatttaatgtacatactaatcgtgaatagtgaatatgatgaaacattgtatcttattgtataaatatccataaacacatcatgaaagacactttctttcacggtctgaattaattatgatacaattctaatagaaaacgaattaaattacgttgaattgtatgaaatctaattgaacaagccaaccacgacgacgactaacgttgcctggattgactcggtttaagttaaccactaaaaaaacggagctgtcatgtaacacgcggatcgagcaggtcacagtcatgaagccatcaaagcaaaagaactaatccaagggctgagatgattaattagtttaaaaattagttaacacgagggaaaaggctgtctgacagccaggtcacgttatctttacctgtggtcgaaatgattcgtgtctgtcgattttaattatttttttgaaaggccgaaaataaagttgtaagagataaacccgcctatataaattcatatattttctctccgctttgaattgtctcgttgtcctcctcactttcatcggccgtttttgaatctccggcgacttgacagagaagaacaaggaagaagactaagagagaaagtaagagataatccaggagattcattctccgttttgaatcttcctcaatctcatcttcttccgctctttctttccaaggtaataggaactttctggatctactttatttgctggatctcgatcttgttttctcaatttccttgagatttggaattcgtttaatttggatctgtgaacctccactaaatcttttggttttactagaatcgatctaagttgaccgatcagttagctcgattatagctaccagaatttggcttgaccttgatggagagatccatgttcatgttacctgggaaatgatttgtatatgtgaattgaaatctgaactgttgaagttagattgaatctgaacactgtcaatgttagattgaatctgaacactgtttaaggttagatgaagtttgtgtatagattcttcgaaactttaggatttgtagtgtcgtacgttgaacagaaagctatttctgattcaatcagggtttatttgactgtattgaactctttttgtgtgtttgcagcagatctacaatggcgcaagttagcagaatctgcaatggtgtgcagaacccatctcttatctccaatctctcgaaatccagtcaacgcaaatctcccttatcggtttctctgaagacgcagcagcatccacgagcttatccgatttcgtcgtcgtggggattgaagaagagtgggatgacgttaattggctctgagcttcgtcctcttaaggtcatgtcttctgtttccacggcgtgcatgcttgccatggataactcagttttgaacagtgggagaactacaatctgtgatgcttataacgtggcagctcatgaccctttttcttttcagcacaagagtcttgatactgtccaaaaggagtggacagaatggaaaaagaataaccactctctttacttggaccctattgtgggtactgtcgcctccttcctccttaaaaaagttggatcactcgttggaaagagaattttgagtgagttgagaaatcttattttcccttcaggatctaccaatttgatgcaagacattctcagggagactgaaaaatttctcaaccagaggcttaacactgacaccctcgccagagtgaatgctgagcttactggcttgcaagctaatgttgaggagtttaacaggcaagtcgataatttcctcaatccaaacagaaacgctgtgcccctcagcataacttcatcagtgaacactatgcaacaactgtttttgaatagattgccccagtttcagatgcaaggttaccaactcctcttgcttccactcttcgcccaggctgctaacctgcatctcagttttatcagggatgtgattttgaatgctgatgagtgggggatttcagctgccacccttaggacctaccgcgattatctcaaaaactacactagggactactctaattactgcattaacacttatcagagcgctttcaagggacttaataccagactgcacgacatgctcgagtttaggacttacatgtttctgaatgttttcgagtacgtcagtatttggagtcttttcaagtatcagtcactccttgttagcagcggtgctaacttgtacgcttctgggtcagggccccagcagactcagagctttacaagccaggattggcccttcctgtattctctgtttcaagtgaatagtaattacgtgttgaacggtttctccggggctaggctgtcaaatacctttcccaacattgtgggacttcctggatctactaccactcacgctctcctggcagctagggttaattattctggcggcattagtagcggagatattggggcttctccattcaatcagaatttcaactgttctacttttcttcctccactccttactcccttcgttagatcctggttggatagtgggtctgatagagagggcgtcgccaccgttacaaactggcaaaccgaatcctttgaaacaacactcggacttaggtctggcgctttcacagctagaggaaattccaattactttcctgattattttattaggaacataagtggcgttccactcgttgttaggaatgaggacctgaggagacctcttcattacaacgaaataagaaacatcgcatctccatcaggcacccctggcggagctagggcttatatggtttccgtgcataatagaaagaacaacattcatgctgtccacgagaatggatcaatgattcacctggctcccaacgactataccgggtttactatttcacctattcacgccacacaagtcaacaatcagacaaggaccttcatttccgagaaattcggaaatcagggggacagtctgagattcgagcagaataacactaccgcaagatatactcttagaggaaatggaaattcttacaacttgtacttgagggtgagctcaatcggcaattcaacaatcagagttactattaacggcagggtgtatactgcaacaaacgtcaacactactacaaacaatgatggcgttaatgataacggagcaaggttctcagatattaacattgggaatgttgtcgcaagttccaattcagatgtgccccttgatattaacgtgacacttaattcaggcacccaatttgacttgatgaacataatgctggtgcccacaaatatctcaccactctactaataaggccaaggcgatctatgactgaattgccaatgcaccagcctgtctacatgatgaataaataaagagtccatccagtgtgatggctcatgcctgtgtgagtgtgactgaatccatcagtgtgtgtgtgtgtttgtgtcaaccatgtgtgaatcaggtgtcaaaaatcgtggctggaaatccatgtggtttctagctttatgtaaatgttgtttgtgaaatataaatattgttttgtgtatgtgaattttactctctcatttttctcttgcactcaccattctattatagtaatttttttaatcgccagcagaacacgcgctgaggcaaatcctaccacctcatttgcaaatttattatgtgttttttttccgtggtcgagattgtgtattattctttagttattacaagacttttagctaaaatttgaaagaatttactttaagaaaatcttaacatctgagataatttcagcaatagattatatttttcattactctagcagtatttttgcagatcaatcgcaacatatatggttgttagaaaaaatgcactatatatatatatattattttttcaattaaaagtgcatgatatataatatatatatatatatatatgtgtgtgtgtatatggtcaaagaaattcttatacaaatatacacgaacacatatatttgacaaaatcaaagtattacactaaacaatgagttggtgcatggccaaaacaaatatgtagattaaaaattccagcctccaaaaaaaaatccaagtgttgtaaagcattatatatatatagtagatcccaaatttttgtacaattccacactgatcgaatttttaaagttgaatatctgacgtaggatttttttaatgtcttacctgaccatttactaataacattcatacgttttcatttgaaatatcctctataattatattgaatttggcacataataagaaacctaattggtgatttattttactagtaaatttctggtgatgggctttctactagaaagctctcggaaaatcttggaccaaatccatattccatgacttcgattgttaaccctattagttttcacaaacatactatcaatatcattgcaacggaaaaggtacaagtaaaacattcaatccgatagggaagtgatgtaggaggttgggaagacaggcccagaaagagatttatctgacttgttttgtgtatagttttcaatgttcataaaggaagatggagacttgagaagttttttttggactttgtttagctttgttgggcgtttttttttttgatcaataactttgttgggcttatgatttgtaatattttcgtggactctttagtttatttagacgtgctaactttgttgggcttatgacttgttgtaacatattgtaacagatgacttgatgtgcgactaatctttacacattaaacatagttctgttttttgaaagttcttattttcatttttatttgaatgttatatatttttctatatttataattctagtaaaaggcaaattttgcttttaaatgaaaaaaatatatattccacagtttcacctaatcttatgcatttagcagtacaaattcaaaaatttcccatttttattcatgaatcataccattatatattaactaaatccaaggtaaaaaaaaggtatgaaagctctatagtaagtaaaatataaattccccataaggaaagggccaagtccaccaggcaagtaaaatgagcaagcaccactccaccatcacacaatttcactcatagataacgataagattcatggaattatcttccacgtggcattattccagcggttcaagccgataagggtctcaacacctctccttaggcctttgtggccgttaccaagtaaaattaacctcacacatatccacactcaaaatccaacggtgtagatcctagtccacttgaatctcatgtatcctagaccctccgatcactccaaagcttgttctcattgttgttatcattatatatagatgaccaaagcactagaccaaacctcagtcacacaaagagtaaagaagaacaatggcttcctctatgctctcttccgctactatggttgcctctccggctcaggccactatggtcgctcctttcaacggacttaagtcctccgctgccttcccagccacccgcaaggctaacaacgacattacttccatcacaagcaacggcggaagagttaactgcatgcaggtgtggcctccgattggaaagaagaagtttgagactctctcttaccttcctgaccttaccgattccggtggtcgcgtcaactgcatgcaggccatggacaacaacccaaacatcaacgaatgcattccatacaactgcttgagtaacccagaagttgaagtacttggtggagaacgcattgaaaccggttacactcccatcgacatctccttgtccttgacacagtttctgctcagcgagttcgtgccaggtgctgggttcgttctcggactagttgacatcatctggggtatctttggtccatctcaatgggatgcattcctggtgcaaattgagcagttgatcaaccagaggatcgaagagttcgccaggaaccaggccatctctaggttggaaggattgagcaatctctaccaaatctatgcagagagcttcagagagtgggaagccgatcctactaacccagctctccgcgaggaaatgcgtattcaattcaacgacatgaacagcgccttgaccacagctatcccattgttcgcagtccagaactaccaagttcctctcttgtccgtgtacgttcaagcagctaatcttcacctcagcgtgcttcgagacgttagcgtgtttgggcaaaggtggggattcgatgctgcaaccatcaatagccgttacaacgaccttactaggctgattggaaactacaccgaccacgctgttcgttggtacaacactggcttggagcgtgtctggggtcctgattctagagattggattagatacaaccagttcaggagagaattgaccctcacagttttggacattgtgtctctcttcccgaactatgactccagaacctaccctatccgtacagtgtcccaacttaccagagaaatctatactaacccagttcttgagaacttcgacggtagcttccgtggttctgcccaaggtatcgaaggctccatcaggagcccacacttgatggacatcttgaacagcataactatctacaccgatgctcacagaggagagtattactggtctggacaccagatcatggcctctccagttggattcagcgggcccgagtttacctttcctctctatggaactatgggaaacgccgctccacaacaacgtatcgttgctcaactaggtcagggtgtctacagaaccttgtcttccaccttgtacagaagacccttcaatatcggtatcaacaaccagcaactttccgttcttgacggaacagagttcgcctatggaacctcttctaacttgccatccgctgtttacagaaagagcggaaccgttgattccttggacgaaatcccaccacagaacaacaatgtgccacccaggcaaggattctcccacaggttgagccacgtgtccatgttccgttccggattcagcaacagttccgtgagcatcatcagagctcctatgttctcttggatacaccgtagtgctgagttcaacaacatcattgcatccgacagcattactcaaatacccttggtgaaagcacatacacttcagtcaggtactactgttgtcagaggtccagggtttacaggaggagacattcttcgtcgcacaagtggaggaccctttgcttacactattgttaacatcaatggccaattgccccaaaggtatcgtgcaagaatccgctatgcctctactacaaatctcaggatctacgtgactgttgcaggtgaaaggatctttgctggtcagttcaacaagactatggataccggtgaccctttgacattccaatcttttagctacgcaactatcaacacagcttttacattcccaatgagccagagtagcttcacagtaggtgctgacactttcagctcagggaatgaagtttacatcgacaggtttgaattgattccagttactgcaaccctcgaggctgagtacaaccttgagagagcccagaaggctgtgaacgccctctttacctccaccaatcagcttggcttgaaaactaacgttactgactatcacattgaccaagtgtccaacttggtcacctaccttagcgatgagttctgcctcgacgagaagcgtgaactctccgagaaagttaaacacgccaagcgtctcagcgacgagaggaatctcttgcaagactccaacttcaaagacatcaacaggcagccagaacgtggttggggtggaagcaccgggatcaccatccaaggaggcgacgatgtgttcaaggagaactacgtcaccctctccggaactttcgacgagtgctaccctacctacttgtaccagaagatcgatgagtccaaactcaaagccttcaccaggtatcaacttagaggctacatcgaagacagccaagaccttgaaatctactcgatcaggtacaatgccaagcacgagaccgtgaatgtcccaggtactggttccctctggccactttctgcccaatctcccattgggaagtgtggagagcctaacagatgcgctccacaccttgagtggaatcctgacttggactgctcctgcagggatggcgagaagtgtgcccaccattctcatcacttctccttggacatcgatgtgggatgtactgacctgaatgaggacctcggagtctgggtcatcttcaagatcaagacccaagacggacacgcaagacttggcaaccttgagtttctcgaagagaaaccattggtcggtgaagctctcgctcgtgtgaagagagcagagaagaagtggagggacaaacgtgagaaactcgaatgggaaactaacatcgtttacaaggaggccaaagagtccgtggatgctttgttcgtgaactcccaatatgatcagttgcaagccgacaccaacatcgccatgatccacgccgcagacaaacgtgtgcacagcattcgtgaggcttacttgcctgagttgtccgtgatccctggtgtgaacgctgccatcttcgaggaacttgagggacgtatctttaccgcattctccttgtacgatgccagaaacgtcatcaagaacggtgacttcaacaatggcctcagctgctggaatgtgaaaggtcatgtggacgtggaggaacagaacaatcagcgttccgtcctggttgtgcctgagtgggaagctgaagtgtcccaagaggttagagtctgtccaggtagaggctacattctccgtgtgaccgcttacaaggagggatacggtgagggttgcgtgaccatccacgagatcgagaacaacaccgacgagcttaagttctccaactgcgtcgaggaagaaatctatcccaacaacaccgttacttgcaacgactacactgtgaatcaggaagagtacggaggtgcctacactagccgtaacagaggttacaacgaagctccttccgttcctgctgactatgcctccgtgtacgaggagaaatcctacacagatggcagacgtgagaacccttgcgagttcaacagaggttacagggactacacaccacttccagttggctatgttaccaaggagcttgagtactttcctgagaccgacaaagtgtggatcgagatcggtgaaaccgagggaaccttcatcgtggacagcgtggagcttctcttgatggaggaataatgagcaaggaggatcatgaacatcacaaagtgaatttattttatgtttgcaccatatattattatttgtgacacattttagaactcttaaaccatttttctgtttgcattttagctactggttgttgtattcacaataatgatgcagtcctatgcttcttggtgtaagattcaatactatgtaaagtgtatgtctttggttgtatactatttaaaatctattcttgtattgtataatttattttagcctttgtttgagattgaggttacttgttctgttgcatttaatcacaagttttcattttgttatacgtacgtgttataccctgtttttggacctaaaaatactgggcccaatttcatttcaaactttgtcaattatcaaatttcaactgcacagttcacaaatagagtgaggttgatttgcggccgcacgtcctgcttggcctactaggccaacgcaggcgctggccgtgacggccacgagcgaactaggccttgggccgcatcgatcgtgaagtttctcatctaagcccccatttggacgtgaatgtagacacgtcgaaataaagatttccgaattagaataatttgtttattgctttcgcctataaatacgacggatcgtaatttgtcgttttatcaaaatgtactttcattttataataacgctgcggacatctacatttttgaattgaaaaaaaattggtaattactctttctttttctccatattgaccatcatactcattgctgatccatgtagatt

SEQ ID NO: 10 - DNA, 12640 bp, Artificial Sequence
  Artificial DNA sequence comprising soybean genomic sequence and transgene sequence
ttaatttttaagtaaactaatttatgtctaaagggtttattttaaaaataggttaataataaaatttcatatgatttttttatcaaacacaaaaattatttaaaattaatttaaatttaaattaattttagactaaaaaataatttatcaatatgaagcctaatatgtgaatattaccctatatttacatcttaagtatgtgagttaggtttactaatattatatttcataggtcttttttgttgattttatacatatttcttttcatataaataataacgtttttttatcgtaattattaattttttatttttattaacaggaattcgaagtcatatttatttctttctcgtttagatagcaacttaatgttatgtatttccgttaatacatttttaaaaaaatttacgatattatgataagtcatgatcaaatacgaaacatacttagtgtaacgtcattaaattccatttccatggaatgtgagtacagttcattatttaatttaattttttttttgttgcagaatttaattgaccaggttttgtggtgacgtctctgcacaggcttcccgtaaggcgtcctaatcataatcttaaaattcttcaatatctaccttgtattttgggtaatgggaaaatcagactcgatctgtattttcagttgcaattctcttccttctcgtgactctccagtaccttgttgatttgaacgacttggttaatctttaaattaccttcattaaacattcgtttgaattaggtgttacattgttaggaccacaacggtgtgacctcacaaccttgcggagttaattatggtggattggtgggtacatatatagactcatcatcaggaacaaaaaatatctacgaaaccattatatttatttttgttgtttgagactgtctacatgaatgatacgagactaaagattgttatttgtcaggaattgtaatttatttttactacaatataaacaacgagaaaaacaacggttaggttgacatggtaatcaactaattgtatttaaaaaaaaaaaaaaaaacaattgtaccatcgtacttggctcatgagatccccacatgcttagatcagggcaatccttaactatcactcatgaactcagtcacgacacatagaggaatagttagcgaatgtgactcgaacattgcacgactcccatgacacctgatatgtatatatagatccagatgagagactcacacgtacattttactcatcccaattataaatacataaacactatagaacaccactaaattgctctttggagtttattttgtagatatttcccctcactttggagatctccagtcagcatcatcacaccaaaagttaggcccgaatagtttgaaattagaaagctcgcaattgaggtctgtcgaccctgcaggtacactggcgcgccacctcagcgctgtgcctgttgcgacaactatttttatgtatgcaagagtcagcatatgtataattgattcagaatcgttttgacgagttcggatgtagtagtagccattatttaatgtacatactaatcgtgaatagtgaatatgatgaaacattgtatcttattgtataaatatccataaacacatcatgaaagacactttctttcacggtctgaattaattatgatacaattctaatagaaaacgaattaaattacgttgaattgtatgaaatctaattgaacaagccaaccacgacgacgactaacgttgcctggattgactcggtttaagttaaccactaaaaaaacggagctgtcatgtaacacgcggatcgagcaggtcacagtcatgaagccatcaaagcaaaagaactaatccaagggctgagatgattaattagtttaaaaattagttaacacgagggaaaaggctgtctgacagccaggtcacgttatctttacctgtggtcgaaatgattcgtgtctgtcgattttaattatttttttgaaaggccgaaaataaagttgtaagagataaacccgcctatataaattcatatattttctctccgctttgaattgtctcgttgtcctcctcactttcatcggccgtttttgaatctccggcgacttgacagagaagaacaaggaagaagactaagagagaaagtaagagataatccaggagattcattctccgttttgaatcttcctcaatctcatcttcttccgctctttctttccaaggtaataggaactttctggatctactttatttgctggatctcgatcttgttttctcaatttccttgagatttggaattcgtttaatttggatctgtgaacctccactaaatcttttggttttactagaatcgatctaagttgaccgatcagttagctcgattatagctaccagaatttggcttgaccttgatggagagatccatgttcatgttacctgggaaatgatttgtatatgtgaattgaaatctgaactgttgaagttagattgaatctgaacactgtcaatgttagattgaatctgaacactgtttaaggttagatgaagtttgtgtatagattcttcgaaactttaggatttgtagtgtcgtacgttgaacagaaagctatttctgattcaatcagggtttatttgactgtattgaactctttttgtgtgtttgcagcagatctacaatggcgcaagttagcagaatctgcaatggtgtgcagaacccatctcttatctccaatctctcgaaatccagtcaacgcaaatctcccttatcggtttctctgaagacgcagcagcatccacgagcttatccgatttcgtcgtcgtggggattgaagaagagtgggatgacgttaattggctctgagcttcgtcctcttaaggtcatgtcttctgtttccacggcgtgcatgcttgccatggataactcagttttgaacagtgggagaactacaatctgtgatgcttataacgtggcagctcatgaccctttttcttttcagcacaagagtcttgatactgtccaaaaggagtggacagaatggaaaaagaataaccactctctttacttggaccctattgtgggtactgtcgcctccttcctccttaaaaaagttggatcactcgttggaaagagaattttgagtgagttgagaaatcttattttcccttcaggatctaccaatttgatgcaagacattctcagggagactgaaaaatttctcaaccagaggcttaacactgacaccctcgccagagtgaatgctgagcttactggcttgcaagctaatgttgaggagtttaacaggcaagtcgataatttcctcaatccaaacagaaacgctgtgcccctcagcataacttcatcagtgaacactatgcaacaactgtttttgaatagattgccccagtttcagatgcaaggttaccaactcctcttgcttccactcttcgcccaggctgctaacctgcatctcagttttatcagggatgtgattttgaatgctgatgagtgggggatttcagctgccacccttaggacctaccgcgattatctcaaaaactacactagggactactctaattactgcattaacacttatcagagcgctttcaagggacttaataccagactgcacgacatgctcgagtttaggacttacatgtttctgaatgttttcgagtacgtcagtatttggagtcttttcaagtatcagtcactccttgttagcagcggtgctaacttgtacgcttctgggtcagggccccagcagactcagagctttacaagccaggattggcccttcctgtattctctgtttcaagtgaatagtaattacgtgttgaacggtttctccggggctaggctgtcaaatacctttcccaacattgtgggacttcctggatctactaccactcacgctctcctggcagctagggttaattattctggcggcattagtagcggagatattggggcttctccattcaatcagaatttcaactgttctacttttcttcctccactccttactcccttcgttagatcctggttggatagtgggtctgatagagagggcgtcgccaccgttacaaactggcaaaccgaatcctttgaaacaacactcggacttaggtctggcgctttcacagctagaggaaattccaattactttcctgattattttattaggaacataagtggcgttccactcgttgttaggaatgaggacctgaggagacctcttcattacaacgaaataagaaacatcgcatctccatcaggcacccctggcggagctagggcttatatggtttccgtgcataatagaaagaacaacattcatgctgtccacgagaatggatcaatgattcacctggctcccaacgactataccgggtttactatttcacctattcacgccacacaagtcaacaatcagacaaggaccttcatttccgagaaattcggaaatcagggggacagtctgagattcgagcagaataacactaccgcaagatatactcttagaggaaatggaaattcttacaacttgtacttgagggtgagctcaatcggcaattcaacaatcagagttactattaacggcagggtgtatactgcaacaaacgtcaacactactacaaacaatgatggcgttaatgataacggagcaaggttctcagatattaacattgggaatgttgtcgcaagttccaattcagatgtgccccttgatattaacgtgacacttaattcaggcacccaatttgacttgatgaacataatgctggtgcccacaaatatctcaccactctactaataaggccaaggcgatctatgactgaattgccaatgcaccagcctgtctacatgatgaataaataaagagtccatccagtgtgatggctcatgcctgtgtgagtgtgactgaatccatcagtgtgtgtgtgtgtttgtgtcaaccatgtgtgaatcaggtgtcaaaaatcgtggctggaaatccatgtggtttctagctttatgtaaatgttgtttgtgaaatataaatattgttttgtgtatgtgaattttactctctcatttttctcttgcactcaccattctattatagtaatttttttaatcgccagcagaacacgcgctgaggcaaatcctaccacctcatttgcaaatttattatgtgttttttttccgtggtcgagattgtgtattattctttagttattacaagacttttagctaaaatttgaaagaatttactttaagaaaatcttaacatctgagataatttcagcaatagattatatttttcattactctagcagtatttttgcagatcaatcgcaacatatatggttgttagaaaaaatgcactatatatatatatattattttttcaattaaaagtgcatgatatataatatatatatatatatatatgtgtgtgtgtatatggtcaaagaaattcttatacaaatatacacgaacacatatatttgacaaaatcaaagtattacactaaacaatgagttggtgcatggccaaaacaaatatgtagattaaaaattccagcctccaaaaaaaaatccaagtgttgtaaagcattatatatatatagtagatcccaaatttttgtacaattccacactgatcgaatttttaaagttgaatatctgacgtaggatttttttaatgtcttacctgaccatttactaataacattcatacgttttcatttgaaatatcctctataattatattgaatttggcacataataagaaacctaattggtgatttattttactagtaaatttctggtgatgggctttctactagaaagctctcggaaaatcttggaccaaatccatattccatgacttcgattgttaaccctattagttttcacaaacatactatcaatatcattgcaacggaaaaggtacaagtaaaacattcaatccgatagggaagtgatgtaggaggttgggaagacaggcccagaaagagatttatctgacttgttttgtgtatagttttcaatgttcataaaggaagatggagacttgagaagttttttttggactttgtttagctttgttgggcgtttttttttttgatcaataactttgttgggcttatgatttgtaatattttcgtggactctttagtttatttagacgtgctaactttgttgggcttatgacttgttgtaacatattgtaacagatgacttgatgtgcgactaatctttacacattaaacatagttctgttttttgaaagttcttattttcatttttatttgaatgttatatatttttctatatttataattctagtaaaaggcaaattttgcttttaaatgaaaaaaatatatattccacagtttcacctaatcttatgcatttagcagtacaaattcaaaaatttcccatttttattcatgaatcataccattatatattaactaaatccaaggtaaaaaaaaggtatgaaagctctatagtaagtaaaatataaattccccataaggaaagggccaagtccaccaggcaagtaaaatgagcaagcaccactccaccatcacacaatttcactcatagataacgataagattcatggaattatcttccacgtggcattattccagcggttcaagccgataagggtctcaacacctctccttaggcctttgtggccgttaccaagtaaaattaacctcacacatatccacactcaaaatccaacggtgtagatcctagtccacttgaatctcatgtatcctagaccctccgatcactccaaagcttgttctcattgttgttatcattatatatagatgaccaaagcactagaccaaacctcagtcacacaaagagtaaagaagaacaatggcttcctctatgctctcttccgctactatggttgcctctccggctcaggccactatggtcgctcctttcaacggacttaagtcctccgctgccttcccagccacccgcaaggctaacaacgacattacttccatcacaagcaacggcggaagagttaactgcatgcaggtgtggcctccgattggaaagaagaagtttgagactctctcttaccttcctgaccttaccgattccggtggtcgcgtcaactgcatgcaggccatggacaacaacccaaacatcaacgaatgcattccatacaactgcttgagtaacccagaagttgaagtacttggtggagaacgcattgaaaccggttacactcccatcgacatctccttgtccttgacacagtttctgctcagcgagttcgtgccaggtgctgggttcgttctcggactagttgacatcatctggggtatctttggtccatctcaatgggatgcattcctggtgcaaattgagcagttgatcaaccagaggatcgaagagttcgccaggaaccaggccatctctaggttggaaggattgagcaatctctaccaaatctatgcagagagcttcagagagtgggaagccgatcctactaacccagctctccgcgaggaaatgcgtattcaattcaacgacatgaacagcgccttgaccacagctatcccattgttcgcagtccagaactaccaagttcctctcttgtccgtgtacgttcaagcagctaatcttcacctcagcgtgcttcgagacgttagcgtgtttgggcaaaggtggggattcgatgctgcaaccatcaatagccgttacaacgaccttactaggctgattggaaactacaccgaccacgctgttcgttggtacaacactggcttggagcgtgtctggggtcctgattctagagattggattagatacaaccagttcaggagagaattgaccctcacagttttggacattgtgtctctcttcccgaactatgactccagaacctaccctatccgtacagtgtcccaacttaccagagaaatctatactaacccagttcttgagaacttcgacggtagcttccgtggttctgcccaaggtatcgaaggctccatcaggagcccacacttgatggacatcttgaacagcataactatctacaccgatgctcacagaggagagtattactggtctggacaccagatcatggcctctccagttggattcagcgggcccgagtttacctttcctctctatggaactatgggaaacgccgctccacaacaacgtatcgttgctcaactaggtcagggtgtctacagaaccttgtcttccaccttgtacagaagacccttcaatatcggtatcaacaaccagcaactttccgttcttgacggaacagagttcgcctatggaacctcttctaacttgccatccgctgtttacagaaagagcggaaccgttgattccttggacgaaatcccaccacagaacaacaatgtgccacccaggcaaggattctcccacaggttgagccacgtgtccatgttccgttccggattcagcaacagttccgtgagcatcatcagagctcctatgttctcttggatacaccgtagtgctgagttcaacaacatcattgcatccgacagcattactcaaatacccttggtgaaagcacatacacttcagtcaggtactactgttgtcagaggtccagggtttacaggaggagacattcttcgtcgcacaagtggaggaccctttgcttacactattgttaacatcaatggccaattgccccaaaggtatcgtgcaagaatccgctatgcctctactacaaatctcaggatctacgtgactgttgcaggtgaaaggatctttgctggtcagttcaacaagactatggataccggtgaccctttgacattccaatcttttagctacgcaactatcaacacagcttttacattcccaatgagccagagtagcttcacagtaggtgctgacactttcagctcagggaatgaagtttacatcgacaggtttgaattgattccagttactgcaaccctcgaggctgagtacaaccttgagagagcccagaaggctgtgaacgccctctttacctccaccaatcagcttggcttgaaaactaacgttactgactatcacattgaccaagtgtccaacttggtcacctaccttagcgatgagttctgcctcgacgagaagcgtgaactctccgagaaagttaaacacgccaagcgtctcagcgacgagaggaatctcttgcaagactccaacttcaaagacatcaacaggcagccagaacgtggttggggtggaagcaccgggatcaccatccaaggaggcgacgatgtgttcaaggagaactacgtcaccctctccggaactttcgacgagtgctaccctacctacttgtaccagaagatcgatgagtccaaactcaaagccttcaccaggtatcaacttagaggctacatcgaagacagccaagaccttgaaatctactcgatcaggtacaatgccaagcacgagaccgtgaatgtcccaggtactggttccctctggccactttctgcccaatctcccattgggaagtgtggagagcctaacagatgcgctccacaccttgagtggaatcctgacttggactgctcctgcagggatggcgagaagtgtgcccaccattctcatcacttctccttggacatcgatgtgggatgtactgacctgaatgaggacctcggagtctgggtcatcttcaagatcaagacccaagacggacacgcaagacttggcaaccttgagtttctcgaagagaaaccattggtcggtgaagctctcgctcgtgtgaagagagcagagaagaagtggagggacaaacgtgagaaactcgaatgggaaactaacatcgtttacaaggaggccaaagagtccgtggatgctttgttcgtgaactcccaatatgatcagttgcaagccgacaccaacatcgccatgatccacgccgcagacaaacgtgtgcacagcattcgtgaggcttacttgcctgagttgtccgtgatccctggtgtgaacgctgccatcttcgaggaacttgagggacgtatctttaccgcattctccttgtacgatgccagaaacgtcatcaagaacggtgacttcaacaatggcctcagctgctggaatgtgaaaggtcatgtggacgtggaggaacagaacaatcagcgttccgtcctggttgtgcctgagtgggaagctgaagtgtcccaagaggttagagtctgtccaggtagaggctacattctccgtgtgaccgcttacaaggagggatacggtgagggttgcgtgaccatccacgagatcgagaacaacaccgacgagcttaagttctccaactgcgtcgaggaagaaatctatcccaacaacaccgttacttgcaacgactacactgtgaatcaggaagagtacggaggtgcctacactagccgtaacagaggttacaacgaagctccttccgttcctgctgactatgcctccgtgtacgaggagaaatcctacacagatggcagacgtgagaacccttgcgagttcaacagaggttacagggactacacaccacttccagttggctatgttaccaaggagcttgagtactttcctgagaccgacaaagtgtggatcgagatcggtgaaaccgagggaaccttcatcgtggacagcgtggagcttctcttgatggaggaataatgagcaaggaggatcatgaacatcacaaagtgaatttattttatgtttgcaccatatattattatttgtgacacattttagaactcttaaaccatttttctgtttgcattttagctactggttgttgtattcacaataatgatgcagtcctatgcttcttggtgtaagattcaatactatgtaaagtgtatgtctttggttgtatactatttaaaatctattcttgtattgtataatttattttagcctttgtttgagattgaggttacttgttctgttgcatttaatcacaagttttcattttgttatacgtacgtgttataccctgtttttggacctaaaaatactgggcccaatttcatttcaaactttgtcaattatcaaatttcaactgcacagttcacaaatagagtgaggttgatttgcggccgcacgtcctgcttggcctactaggccaacgcaggcgctggccgtgacggccacgagcgaactaggccttgggccgcatcgatcgtgaagtttctcatctaagcccccatttggacgtgaatgtagacacgtcgaaataaagatttccgaattagaataatttgtttattgctttcgcctataaatacgacggatcgtaatttgtcgttttatcaaaatgtactttcattttataataacgctgcggacatctacatttttgaattgaaaaaaaattggtaattactctttctttttctccatattgaccatcatactcattgctgatccatgtagattcctatgagaatgagaggacaagacagctcggtcaaaactcaatcgtcgaaattcaatgggaacattttggtatctaacctcaacttcaatactggagatcggaaattccactaacaaggaaatgaccattcgatcggacctcatcagaactcagtagtaacatattgtatttgaaagaacaattaaatcatatataagcttttgtggaaaaaaaggatactacgtactaaaatataaacgttgaagtaaattacagaaaatgctaatttcataacacggttatcttcaaattttagtggcccgtttaagccctagttaaatcaaatatatgaatgcagtttatgtataaggtatgcatgtgttatagttaatcgagtttagataattagaatcaaatatatgattaatggtacctgtgttacataaagagactaattaacctaagttctgaacaagtaattaatcaaacattgaagtgatagatgttgggcctaaatccagagcataacctttacgtcaatgaactacaaattttcacactagaaacatacattgaactttttttccttcgtttaaactccttttcttttaactgtgtttccgcgtttaatcaaattttacgtgtgtcgaccgaaagttagaaattataactaataacagactcaagttgacgtaattttttcatgatacctacgtattgctcggagtttagatgctatataaacatgagtgatgacatggttttaaattgtgcttccagttgtgttaccatgaactaaaaaatcttataggtaattgtaagaaaatatgattgatccagtcatgattgcggttatgatgcgattgtacagaatcaaaataccttgaaattgcgattgcaattgttattacagactccaatttaaaatcatgagtgaggattttatgatagatcgaatcaatgtttcacactacacctggaataaaaacctgagtcgtttattagatctatatcttcatatgcatgcatgtaccttagctattcatttttcactgtaaatctttactcacacttaaaatagtcgtgcatttgatatttgaatgaaatttatagagctttcgatttgagatagtcccatctctatttgggttggtcaatcatggagcatgaaaaaaacaatagtttagctaggccaggccaaattaat

SEQ ID NO: 11 - DNA, 27 bp, Artificial Sequence
  Chemically Synthesized Oligonucleotide PCR Primer
ctctttctttttctccatattgaccat

SEQ ID NO: 12 - DNA, 26 bp, Artificial Sequence
  Chemically Synthesized Oligonucleotide PCR Primer
ctgtcttgtcctctcattctcatagg

SEQ ID NO: 13 - DNA, 19 bp, Artificial Sequence
  Chemically Synthesized Oligonucleotide PCR Probe
atactcattgctgatccat

SEQ ID NO: 14 - DNA, 24 bp, Artificial Sequence
  Chemically Synthesized Oligonucleotide PCR Primer
agctgtcttgtcctctcattctca

SEQ ID NO: 15 - DNA, 30 bp, Artificial Sequence
  Chemically Synthesized Oligonucleotide PCR Primer
ctctttggagtttattttgtagatatttcc

SEQ ID NO: 16 - DNA, 18 bp, Artificial Sequence
  Chemically Synthesized Oligonucleotide PCR Probe
tcactttggagatcggag

SEQ ID NO: 17 - DNA, 112 bp, Artificial Sequence
  Artificial DNA sequence comprising transgene sequence
atagtttgaaattagaaagctcgcaattgaggtctgtcgaccctgcaggtacactggcgcgccacctcagcgctgtgcctgttgcgacaactatttttatgtatgcaagagt

SEQ ID NO: 18 - DNA, 52 bp, Artificial Sequence
  Artificial DNA sequence comprising transgene sequence
attgaactctttttgtgtgtttgcagcagatctacaatggcgcaagttagca

SEQ ID NO: 19 - DNA, 283 bp, Artificial Sequence
  Artificial DNA sequence comprising transgene sequence
cggcgtgcatgcttgccatggataactcagttttgaacagtgggagaactacaatctgtgatgcttataacgtggcagctcatgaccctttttcttttcagcacaagagtcttgatactgtccaaaaggagtggacagaatggaaaaagaataaccactctctttacttggaccctattgtgggtactgtcgcctccttcctccttaaaaaagttggatcactcgttggaaagagaattttgagtgagttgagaaatcttattttcccttcaggatctaccaa

SEQ ID NO: 20 - DNA, 486 bp, Artificial Sequence
  Artificial DNA sequence comprising transgene sequence
gagtacgtcagtatttggagtcttttcaagtatcagtcactccttgttagcagcggtgctaacttgtacgcttctgggtcagggccccagcagactcagagctttacaagccaggattggcccttcctgtattctctgtttcaagtgaatagtaattacgtgttgaacggtttctccggggctaggctgtcaaatacctttcccaacattgtgggacttcctggatctactaccactcacgctctcctggcagctagggttaattattctggcggcattagtagcggagatattggggcttctccattcaatcagaatttcaactgttctacttttcttcctccactccttactcccttcgttagatcctggttggatagtgggtctgatagagagggcgtcgccaccgttacaaactggcaaaccgaatcctttgaaacaacactcggacttaggtctggcgctttcacagctagaggaaattcc

SEQ ID NO: 21 - DNA, 179 bp, Artificial Sequence
  Artificial DNA sequence comprising transgene sequence
taacggagcaaggttctcagatattaacattgggaatgttgtcgcaagttccaattcagatgtgccccttgatattaacgtgacacttaattcaggcacccaatttgacttgatgaacataatgctggtgcccacaaatatctcaccactctactaataaggccaaggcgatctatgac

SEQ ID NO: 22 - DNA, 106 bp, Artificial Sequence
  Artificial DNA sequence comprising transgene sequence
tcttgcactcaccattctattatagtaatttttttaatcgccagcagaacacgcgctgaggcaaatcctaccacctcatttgcaaatttattatgtgttttttttc

SEQ ID NO: 23 - DNA, 60 bp, Artificial Sequence
  Artificial DNA sequence comprising transgene sequence
acagcgtggagcttctcttgatggaggaataatgagcaaggaggatcatgaacatcacaa

SEQ ID NO: 24 - DNA, 66 bp, Artificial Sequence
  Artificial DNA sequence comprising transgene sequence
cttgttctgttgcatttaatcacaagttttcattttgttatacgtacgtgttataccctgtttttg

SEQ ID NO: 25 - DNA, 156 bp, Artificial Sequence
  Artificial DNA sequence comprising transgene sequence
ctttgtcaattatcaaatttcaactgcacagttcacaaatagagtgaggttgatttgcggccgcacgtcctgcttggcctactaggccaacgcaggcgctggccgtgacggccacgagcgaactaggccttgggccgcatcgatcgtgaagtttct

SEQ ID NO: 26 - DNA, 1905 bp, Artificial Sequence
  Artificial DNA sequence comprising transgene sequence
atggataactcagttttgaacagtgggagaactacaatctgtgatgcttataacgtggcagctcatgaccctttttcttttcagcacaagagtcttgatactgtccaaaaggagtggacagaatggaaaaagaataaccactctctttacttggaccctattgtgggtactgtcgcctccttcctccttaaaaaagttggatcactcgttggaaagagaattttgagtgagttgagaaatcttattttcccttcaggatctaccaatttgatgcaagacattctcagggagactgaaaaatttctcaaccagaggcttaacactgacaccctcgccagagtgaatgctgagcttactggcttgcaagctaatgttgaggagtttaacaggcaagtcgataatttcctcaatccaaacagaaacgctgtgcccctcagcataacttcatcagtgaacactatgcaacaactgtttttgaatagattgccccagtttcagatgcaaggttaccaactcctcttgcttccactcttcgcccaggctgctaacctgcatctcagttttatcagggatgtgattttgaatgctgatgagtgggggatttcagctgccacccttaggacctaccgcgattatctcaaaaactacactagggactactctaattactgcattaacacttatcagagcgctttcaagggacttaataccagactgcacgacatgctcgagtttaggacttacatgtttctgaatgttttcgagtacgtcagtatttggagtcttttcaagtatcagtcactccttgttagcagcggtgctaacttgtacgcttctgggtcagggccccagcagactcagagctttacaagccaggattggcccttcctgtattctctgtttcaagtgaatagtaattacgtgttgaacggtttctccggggctaggctgtcaaatacctttcccaacattgtgggacttcctggatctactaccactcacgctctcctggcagctagggttaattattctggcggcattagtagcggagatattggggcttctccattcaatcagaatttcaactgttctacttttcttcctccactccttactcccttcgttagatcctggttggatagtgggtctgatagagagggcgtcgccaccgttacaaactggcaaaccgaatcctttgaaacaacactcggacttaggtctggcgctttcacagctagaggaaattccaattactttcctgattattttattaggaacataagtggcgttccactcgttgttaggaatgaggacctgaggagacctcttcattacaacgaaataagaaacatcgcatctccatcaggcacccctggcggagctagggcttatatggtttccgtgcataatagaaagaacaacattcatgctgtccacgagaatggatcaatgattcacctggctcccaacgactataccgggtttactatttcacctattcacgccacacaagtcaacaatcagacaaggaccttcatttccgagaaattcggaaatcagggggacagtctgagattcgagcagaataacactaccgcaagatatactcttagaggaaatggaaattcttacaacttgtacttgagggtgagctcaatcggcaattcaacaatcagagttactattaacggcagggtgtatactgcaacaaacgtcaacactactacaaacaatgatggcgttaatgataacggagcaaggttctcagatattaacattgggaatgttgtcgcaagttccaattcagatgtgccccttgatattaacgtgacacttaattcaggcacccaatttgacttgatgaacataatgctggtgcccacaaatatctcaccactctactaa